European Patent Application EP 4 438 726 A2, published October 2, 2024. Title: Compositions and Methods Comprising Plants with Increased Seed Amino Acid Content. Applicant: Benson Hill, Inc. Application US. The sequence listing filed with the application follows.

SEQUENCE LISTING (26 sequences)

SEQ ID NO: 1 - DNA, 4990 bp, Glycine max
  source 1..4990: mol_type = genomic DNA
atgctttctgcaacacttccagtgtcccttacatctgcaaagggctcctccttggccttctcccgccgcatggttccttccggccaccgtctatctccggcgacactcaccggcgtttcactctcacgcgctcctctcacgttgaggtgctcttcactctcaaacaccccttcctatggtaagtgttattttggttttgctagttttgttttgagtaccccacctgaaattataggcagaatgacgaaagggtagctatcctgttcataaaaattcaatcttgttccacgtttaaataaattctacgataactgtgtaaatggtgagtggtggtttgaaagtgctttaactttgaaggcaaaaatgacaaatgggtaggtatctcgattgaaaagttttaatcttttctccgtgtttgaataagttcttcgatatcctgtgtagtaaatgagtatttgtgattttatttatttatttactaaatgatgacttaaatgtgtgtaactgtgaaggcaaaaatgacaattgggtaggtatgttgattgaaaagttttaatctttgctccatgtttgaataaatcttcaatatcctgtggtaaatgggtaggtatcctgttaaatagtgacaatttgattaattttagataagtgaaggagtctgtggctaatgttggtgcttccattcatcagcatttggttaattgcttttgtgttttcaataattataacttttttttttttggttttaatcttggacttaacatgtatgacggatactacttttgcagttgaggaaggaagaaagtttgtagaagcttcaaagaatgggaacttgattcctctctgtcagagcatcttcgctgaccaactcactcctgtccttgcttaccggattttggttaaggaagacgattgggaggctccaagctttcttttagagtctgcagagcctagttatcatgcttcgagtgttgtgagtttgctttttggagtattgtgattttgaattttttgagttgtttgtgtctttaactctttattgaaactgaagacaagattgattgtttattgcaggggcgctatagtgttttaggagcaaacccaactatggaagttgtggcaaaagaaaataaggttacaataattgaccacgaatctgggaatttaactgaggaaattgttgatgatcctatggtgattcccagaaaaatctcagagggttggaaaccctatctcattgatgaactaccagatgcattctgtggtaagagttttatgatcataatgcccgtatttagtaaaacaactttgtgcaacgtctgtatggattactaacgtataacgtgcaacgtctgcatggacaaacaactttgtgataactgaaaatcctaagatagaagagaaaattaaatcgacttgtcgtttatgcttttataatttatagtatctgatgttgacatcttgtggttttagatgattaagattgtcacctgaatcttgctttctgcgttacttgtcgagttgtcgttacttgatgtcttatttatgttatctgtgtgcctgacgcgcagatgcttgtgtgggtgttcacttgcatgtgtgtgaaagacagagggctgtattcttgacgtgttttttcatctaattaacttgtttaagctgctcttctaggtggttgggcaggttatttctcatatgacactgttcgttatgtggaaaagaaaaagctaccattttcaaacgctccagaggatgacaggaaccttgctgacatacatctgggcctctatgagaatgtgattgtgtttgaccatgtagaaaaggtacctgtttttctatgcttcacaagtactgtatcaatgttggcatctagtttggtgtttctcacaagacatttttttgtttctaatgttgacatgtagctcactatttctaatttgcactgtagtatatcctcttatcattttaagaaaaactcaattcagattgcttcataaacaaaatgttatgatttcatttctttcctattgtttttaattggatttttgttcattgaatgaggaacaaaaaatcttttcaatgttcatgtacatgctgttttgacattattggatatataatgatctaattattatttgaagagtagaaatcatgaaatgaccaattactatttaattgcattaatatggattatattcaggattcattcatagcttcaatatttcatgttcactcgtattctgcataacagaaagcatatgtgattctttgggtgagggttgatcggtactcctcggctgagagtgcttataaggatggaatggaaagattagaaaaattagtggccaaattacaagatggccaaccgtaagtcatctattaaccgtttctctctttaatgatgtacctgttatgattgaatcaaaattaatttaaagcatgtgtttcctagcccaaggctggctccaggttctgtggatttacatactcatcattttggtccatctttaaagaagtcaagcatgacaagtgaagcatacaaagaggcagtccttcaggcaaaagaacatattaaagcaggggatattttccagattgtattaagtcagagattcgaacgaagaacatttgctgatccttttgaaatttatagagcattgagagttgttaacccaagtccttatatggcctatttgcaggtttatttctgcgtaacatctgaaacttcttccttcattcaagaaagttttatggttcagctctttcatgttctatgattatgtatttcctaaacaggctaggggatgtattctggttgcttcaagtccagagattcttacacgtgtaaagaaggtaggatttgtacatatattagatttttaaattaaattatacttatacttcttatttggtgactgggatatttgtcataaatcataaataaaaaatatattagactttgttaaattagtctattatttattttaaaacagatagttattatgattttgtcattaacagaataagattatgaaccgtccattggctgggacagctagaagggggaaaacacctgaagaagatgcaaggtttgaagcaatattgctgagagatgaaaagcagtgtgcagagcatgtcatgttggttgatttgggacgcaatgatgttggaaaggtttgttataaatattcaatataatggatactcctatttgtttttttcctgttcaaggtgtcttgaagcaatagcttggtcaattatattgttcatttaaagaaaatactgcctctcttatttcttatattatatttactctataacctcttcaattggagttgacgttttgaacacccacctttcttgtgttaatcccacaagcttctcatccattctcaattcatgatcaagacatcaaaatagaaaatcttgcattgggtttagggataagtaagcttgctttgatgacttccatcatgtcaatgctacactttacttctgtgttacacagctataccccttcccttgccccattgagaaattgaactgactaatactaagttaaaggattaagaaactcaataacactattcttacacaaatggaatcaggccttcttttctttgcacattattcaaagttacatctatcaatatgagtgtttttgtgaaagcaataaaagcaatgcaacggagaagcaacctccatgttgctttggtgtttttgctgggaaagctaaatttctccattgaacatggtttggatgtgttttcaaacacactatatagctaataattggagttcaacaatgctttcattaactgtggttgtcagtccattatctgaacttgtaagggtgttcggtgaaagccaatctgcagttagttatctggttgtgttagaagcagtaggtacatatgtatcttgttaactgctgctttgtggatttgctgtaattaagcgttcttcatttctttgtaacaaatagatatgataatacctcattttgttgtatatcatgatgtagaagaaagtaatttattctgactttttgagaaaatggtttatatttggtattgtgatgattctcgtagcaggagtttctcttttgtaggttgcaaaaagtggttctgtcaaagttgaaaagcttatgaatgttgaacgatattcccatgtcatgcacataagttcaacggtgagaatattttcttgatatcaagtgtgttggtttttcacaaaagatttcttgtaattctggttaccaacacttcccctatattattaaattgatgctgccatggttcctctgtcccaaaaaattatttctctatccaattaagtcagaacactgggtattatttcattgcatttttctgtttaaacaaaaaatgttgcttatttattgtaggttactggagagttgcaagagcatttgactagctgggatgccctgcgagctgcattgcccgttggaactgtcagtggagcaccaaaggtttgtaattttctcgacttctttttagtcaactacgaatgagaaaacgtttttgttttcattttctgttttttacttttaattacaaaactgtttccttacttccaatctatttcctgttttgaaatatgtgttcaaaactttccaccttgattcattcttatgtggatgcaggtgaaggcgatggagttgattgatgagctggaggtgacaaggagggggccttacagtggaggatttggatacatctctttctctggtgagatggacattgctcttgctctcaggacaatggtatttccgagcggaaccaggtatgatacaatgtactcatacaaagacgtcgaccaacgccgcgagtggattgcttaccttcaagccggagctggtatagttgctgacagtgtccctgatgatgagcaccaagagtgtcaaaacaaagctgctggtcttgctcgtgccattgatttggctgagtccgcttttgttgataaatga

SEQ ID NO: 2 - protein, 589 aa, Glycine max
MLSATLPVSLTSAKGSSLAFSRRMVPSGHRLSPATLTGVSLSRAPLTLRCSSLSNTPSYVEEGRKFVEASKNGNLIPLCQSIFADQLTPVLAYRILVKEDDWEAPSFLLESAEPSYHASSVGRYSVLGANPTMEVVAKENKVTIIDHESGNLTEEIVDDPMVIPRKISEGWKPYLIDELPDAFCGGWAGYFSYDTVRYVEKKKLPFSNAPEDDRNLADIHLGLYENVIVFDHVEKKAYVILWVRVDRYSSAESAYKDGMERLEKLVAKLQDGQPPRLAPGSVDLHTHHFGPSLKKSSMTSEAYKEAVLQAKEHIKAGDIFQIVLSQRFERRTFADPFEIYRALRVVNPSPYMAYLQARGCILVASSPEILTRVKKNKIMNRPLAGTARRGKTPEEDARFEAILLRDEKQCAEHVMLVDLGRNDVGKVAKSGSVKVEKLMNVERYSHVMHISSTVTGELQEHLTSWDALRAALPVGTVSGAPKVKAMELIDELEVTRRGPYSGGFGYISFSGEMDIALALRTMVFPSGTRYDTMYSYKDVDQRREWIAYLQAGAGIVADSVPDDEHQECQNKAAGLARAIDLAESAFVDK

SEQ ID NO: 3 - DNA, 4984 bp, synthetic construct
  source 1..4984: mol_type = other DNA
atgctttctgcaacacttccagtgtcccttacatctgcaaagggctcctccttggccttctcccgccgcatggttccttccggccaccgtctatctccggcgacactcaccggcgtttcactctcacgcgctcctctcacgttgaggtgctcttcactctcaaacaccccttcctatggtaagtgttattttggttttgctagttttgttttgagtaccccacctgaaattataggcagaatgacgaaagggtagctatcctgttcataaaaattcaatcttgttccacgtttaaataaattctacgataactgtgtaaatggtgagtggtggtttgaaagtgctttaactttgaaggcaaaaatgacaaatgggtaggtatctcgattgaaaagttttaatcttttctccgtgtttgaataagttcttcgatatcctgtgtagtaaatgagtatttgtgattttatttatttatttactaaatgatgacttaaatgtgtgtaactgtgaaggcaaaaatgacaattgggtaggtatgttgattgaaaagttttaatctttgctccatgtttgaataaatcttcaatatcctgtggtaaatgggtaggtatcctgttaaatagtgacaatttgattaattttagataagtgaaggagtctgtggctaatgttggtgcttccattcatcagcatttggttaattgcttttgtgttttcaataattataacttttttttttttggttttaatcttggacttaacatgtatgacggatactacttttgcagttgaggaaggaagaaagtttgtagaagcttcaaagaatgggaacttgattcctctctgtcagagcatcttcgctgaccaactcactcctgtccttgcttaccggattttggttaaggaagacgattgggaggctccaagctttcttttagagtctgcagagcctcatgcttcgagtgttgtgagtttgctttttggagtattgtgattttgaattttttgagttgtttgtgtctttaactctttattgaaactgaagacaagattgattgtttattgcaggggcgctatagtgttttaggagcaaacccaactatggaagttgtggcaaaagaaaataaggttacaataattgaccacgaatctgggaatttaactgaggaaattgttgatgatcctatggtgattcccagaaaaatctcagagggttggaaaccctatctcattgatgaactaccagatgcattctgtggtaagagttttatgatcataatgcccgtatttagtaaaacaactttgtgcaacgtctgtatggattactaacgtataacgtgcaacgtctgcatggacaaacaactttgtgataactgaaaatcctaagatagaagagaaaattaaatcgacttgtcgtttatgcttttataatttatagtatctgatgttgacatcttgtggttttagatgattaagattgtcacctgaatcttgctttctgcgttacttgtcgagttgtcgttacttgatgtcttatttatgttatctgtgtgcctgacgcgcagatgcttgtgtgggtgttcacttgcatgtgtgtgaaagacagagggctgtattcttgacgtgttttttcatctaattaacttgtttaagctgctcttctaggtggttgggcaggttatttctcatatgacactgttcgttatgtggaaaagaaaaagctaccattttcaaacgctccagaggatgacaggaaccttgctgacatacatctgggcctctatgagaatgtgattgtgtttgaccatgtagaaaaggtacctgtttttctatgcttcacaagtactgtatcaatgttggcatctagtttggtgtttctcacaagacatttttttgtttctaatgttgacatgtagctcactatttctaatttgcactgtagtatatcctcttatcattttaagaaaaactcaattcagattgcttcataaacaaaatgttatgatttcatttctttcctattgtttttaattggatttttgttcattgaatgaggaacaaaaaatcttttcaatgttcatgtacatgctgttttgacattattggatatataatgatctaattattatttgaagagtagaaatcatgaaatgaccaattactatttaattgcattaatatggattatattcaggattcattcatagcttcaatatttcatgttcactcgtattctgcataacagaaagcatatgtgattctttgggtgagggttgatcggtactcctcggctgagagtgcttataaggatggaatggaaagattagaaaaattagtggccaaattacaagatggccaaccgtaagtcatctattaaccgtttctctctttaatgatgtacctgttatgattgaatcaaaattaatttaaagcatgtgtttcctagcccaaggctggctccaggttctgtggatttacatactcatcattttggtccatctttaaagaagtcaagcatgacaagtgaagcatacaaagaggcagtccttcaggcaaaagaacatattaaagcaggggatattttccagattgtattaagtcagagattcgaacgaagaacatttgctgatccttttgaaatttatagagcattgagagttgttaacccaagtccttatatggcctatttgcaggtttatttctgcgtaacatctgaaacttcttccttcattcaagaaagttttatggttcagctctttcatgttctatgattatgtatttcctaaacaggctaggggatgtattctggttgcttcaagtccagagattcttacacgtgtaaagaaggtaggatttgtacatatattagatttttaaattaaattatacttatacttcttatttggtgactgggatatttgtcataaatcataaataaaaaatatattagactttgttaaattagtctattatttattttaaaacagatagttattatgattttgtcattaacagaataagattatgaaccgtccattggctgggacagctagaagggggaaaacacctgaagaagatgcaaggtttgaagcaatattgctgagagatgaaaagcagtgtgcagagcatgtcatgttggttgatttgggacgcaatgatgttggaaaggtttgttataaatattcaatataatggatactcctatttgtttttttcctgttcaaggtgtcttgaagcaatagcttggtcaattatattgttcatttaaagaaaatactgcctctcttatttcttatattatatttactctataacctcttcaattggagttgacgttttgaacacccacctttcttgtgttaatcccacaagcttctcatccattctcaattcatgatcaagacatcaaaatagaaaatcttgcattgggtttagggataagtaagcttgctttgatgacttccatcatgtcaatgctacactttacttctgtgttacacagctataccccttcccttgccccattgagaaattgaactgactaatactaagttaaaggattaagaaactcaataacactattcttacacaaatggaatcaggccttcttttctttgcacattattcaaagttacatctatcaatatgagtgtttttgtgaaagcaataaaagcaatgcaacggagaagcaacctccatgttgctttggtgtttttgctgggaaagctaaatttctccattgaacatggtttggatgtgttttcaaacacactatatagctaataattggagttcaacaatgctttcattaactgtggttgtcagtccattatctgaacttgtaagggtgttcggtgaaagccaatctgcagttagttatctggttgtgttagaagcagtaggtacatatgtatcttgttaactgctgctttgtggatttgctgtaattaagcgttcttcatttctttgtaacaaatagatatgataatacctcattttgttgtatatcatgatgtagaagaaagtaatttattctgactttttgagaaaatggtttatatttggtattgtgatgattctcgtagcaggagtttctcttttgtaggttgcaaaaagtggttctgtcaaagttgaaaagcttatgaatgttgaacgatattcccatgtcatgcacataagttcaacggtgagaatattttcttgatatcaagtgtgttggtttttcacaaaagatttcttgtaattctggttaccaacacttcccctatattattaaattgatgctgccatggttcctctgtcccaaaaaattatttctctatccaattaagtcagaacactgggtattatttcattgcatttttctgtttaaacaaaaaatgttgcttatttattgtaggttactggagagttgcaagagcatttgactagctgggatgccctgcgagctgcattgcccgttggaactgtcagtggagcaccaaaggtttgtaattttctcgacttctttttagtcaactacgaatgagaaaacgtttttgttttcattttctgttttttacttttaattacaaaactgtttccttacttccaatctatttcctgttttgaaatatgtgttcaaaactttccaccttgattcattcttatgtggatgcaggtgaaggcgatggagttgattgatgagctggaggtgacaaggagggggccttacagtggaggatttggatacatctctttctctggtgagatggacattgctcttgctctcaggacaatggtatttccgagcggaaccaggtatgatacaatgtactcatacaaagacgtcgaccaacgccgcgagtggattgcttaccttcaagccggagctggtatagttgctgacagtgtccctgatgatgagcaccaagagtgtcaaaacaaagctgctggtcttgctcgtgccattgatttggctgagtccgcttttgttgataaatga

SEQ ID NO: 4 - DNA, 4978 bp, synthetic construct
  source 1..4978: mol_type = other DNA
atgctttctgcaacacttccagtgtcccttacatctgcaaagggctcctccttggccttctcccgccgcatggttccttccggccaccgtctatctccggcgacactcaccggcgtttcactctcacgcgctcctctcacgttgaggtgctcttcactctcaaacaccccttcctatggtaagtgttattttggttttgctagttttgttttgagtaccccacctgaaattataggcagaatgacgaaagggtagctatcctgttcataaaaattcaatcttgttccacgtttaaataaattctacgataactgtgtaaatggtgagtggtggtttgaaagtgctttaactttgaaggcaaaaatgacaaatgggtaggtatctcgattgaaaagttttaatcttttctccgtgtttgaataagttcttcgatatcctgtgtagtaaatgagtatttgtgattttatttatttatttactaaatgatgacttaaatgtgtgtaactgtgaaggcaaaaatgacaattgggtaggtatgttgattgaaaagttttaatctttgctccatgtttgaataaatcttcaatatcctgtggtaaatgggtaggtatcctgttaaatagtgacaatttgattaattttagataagtgaaggagtctgtggctaatgttggtgcttccattcatcagcatttggttaattgcttttgtgttttcaataattataacttttttttttttggttttaatcttggacttaacatgtatgacggatactacttttgcagttgaggaaggaagaaagtttgtagaagcttcaaagaatgggaacttgattcctctctgtcagagcatcttcgctgaccaactcactcctgtccttgcttaccggattttggttaaggaagacgattgggaggctccaagctttcttttagagtctgcagatgcttcgagtgttgtgagtttgctttttggagtattgtgattttgaattttttgagttgtttgtgtctttaactctttattgaaactgaagacaagattgattgtttattgcaggggcgctatagtgttttaggagcaaacccaactatggaagttgtggcaaaagaaaataaggttacaataattgaccacgaatctgggaatttaactgaggaaattgttgatgatcctatggtgattcccagaaaaatctcagagggttggaaaccctatctcattgatgaactaccagatgcattctgtggtaagagttttatgatcataatgcccgtatttagtaaaacaactttgtgcaacgtctgtatggattactaacgtataacgtgcaacgtctgcatggacaaacaactttgtgataactgaaaatcctaagatagaagagaaaattaaatcgacttgtcgtttatgcttttataatttatagtatctgatgttgacatcttgtggttttagatgattaagattgtcacctgaatcttgctttctgcgttacttgtcgagttgtcgttacttgatgtcttatttatgttatctgtgtgcctgacgcgcagatgcttgtgtgggtgttcacttgcatgtgtgtgaaagacagagggctgtattcttgacgtgttttttcatctaattaacttgtttaagctgctcttctaggtggttgggcaggttatttctcatatgacactgttcgttatgtggaaaagaaaaagctaccattttcaaacgctccagaggatgacaggaaccttgctgacatacatctgggcctctatgagaatgtgattgtgtttgaccatgtagaaaaggtacctgtttttctatgcttcacaagtactgtatcaatgttggcatctagtttggtgtttctcacaagacatttttttgtttctaatgttgacatgtagctcactatttctaatttgcactgtagtatatcctcttatcattttaagaaaaactcaattcagattgcttcataaacaaaatgttatgatttcatttctttcctattgtttttaattggatttttgttcattgaatgaggaacaaaaaatcttttcaatgttcatgtacatgctgttttgacattattggatatataatgatctaattattatttgaagagtagaaatcatgaaatgaccaattactatttaattgcattaatatggattatattcaggattcattcatagcttcaatatttcatgttcactcgtattctgcataacagaaagcatatgtgattctttgggtgagggttgatcggtactcctcggctgagagtgcttataaggatggaatggaaagattagaaaaattagtggccaaattacaagatggccaaccgtaagtcatctattaaccgtttctctctttaatgatgtacctgttatgattgaatcaaaattaatttaaagcatgtgtttcctagcccaaggctggctccaggttctgtggatttacatactcatcattttggtccatctttaaagaagtcaagcatgacaagtgaagcatacaaagaggcagtccttcaggcaaaagaacatattaaagcaggggatattttccagattgtattaagtcagagattcgaacgaagaacatttgctgatccttttgaaatttatagagcattgagagttgttaacccaagtccttatatggcctatttgcaggtttatttctgcgtaacatctgaaacttcttccttcattcaagaaagttttatggttcagctctttcatgttctatgattatgtatttcctaaacaggctaggggatgtattctggttgcttcaagtccagagattcttacacgtgtaaagaaggtaggatttgtacatatattagatttttaaattaaattatacttatacttcttatttggtgactgggatatttgtcataaatcataaataaaaaatatattagactttgttaaattagtctattatttattttaaaacagatagttattatgattttgtcattaacagaataagattatgaaccgtccattggctgggacagctagaagggggaaaacacctgaagaagatgcaaggtttgaagcaatattgctgagagatgaaaagcagtgtgcagagcatgtcatgttggttgatttgggacgcaatgatgttggaaaggtttgttataaatattcaatataatggatactcctatttgtttttttcctgttcaaggtgtcttgaagcaatagcttggtcaattatattgttcatttaaagaaaatactgcctctcttatttcttatattatatttactctataacctcttcaattggagttgacgttttgaacacccacctttcttgtgttaatcccacaagcttctcatccattctcaattcatgatcaagacatcaaaatagaaaatcttgcattgggtttagggataagtaagcttgctttgatgacttccatcatgtcaatgctacactttacttctgtgttacacagctataccccttcccttgccccattgagaaattgaactgactaatactaagttaaaggattaagaaactcaataacactattcttacacaaatggaatcaggccttcttttctttgcacattattcaaagttacatctatcaatatgagtgtttttgtgaaagcaataaaagcaatgcaacggagaagcaacctccatgttgctttggtgtttttgctgggaaagctaaatttctccattgaacatggtttggatgtgttttcaaacacactatatagctaataattggagttcaacaatgctttcattaactgtggttgtcagtccattatctgaacttgtaagggtgttcggtgaaagccaatctgcagttagttatctggttgtgttagaagcagtaggtacatatgtatcttgttaactgctgctttgtggatttgctgtaattaagcgttcttcatttctttgtaacaaatagatatgataatacctcattttgttgtatatcatgatgtagaagaaagtaatttattctgactttttgagaaaatggtttatatttggtattgtgatgattctcgtagcaggagtttctcttttgtaggttgcaaaaagtggttctgtcaaagttgaaaagcttatgaatgttgaacgatattcccatgtcatgcacataagttcaacggtgagaatattttcttgatatcaagtgtgttggtttttcacaaaagatttcttgtaattctggttaccaacacttcccctatattattaaattgatgctgccatggttcctctgtcccaaaaaattatttctctatccaattaagtcagaacactgggtattatttcattgcatttttctgtttaaacaaaaaatgttgcttatttattgtaggttactggagagttgcaagagcatttgactagctgggatgccctgcgagctgcattgcccgttggaactgtcagtggagcaccaaaggtttgtaattttctcgacttctttttagtcaactacgaatgagaaaacgtttttgttttcattttctgttttttacttttaattacaaaactgtttccttacttccaatctatttcctgttttgaaatatgtgttcaaaactttccaccttgattcattcttatgtggatgcaggtgaaggcgatggagttgattgatgagctggaggtgacaaggagggggccttacagtggaggatttggatacatctctttctctggtgagatggacattgctcttgctctcaggacaatggtatttccgagcggaaccaggtatgatacaatgtactcatacaaagacgtcgaccaacgccgcgagtggattgcttaccttcaagccggagctggtatagttgctgacagtgtccctgatgatgagcaccaagagtgtcaaaacaaagctgctggtcttgctcgtgccattgatttggctgagtccgcttttgttgataaatga

SEQ ID NO: 5 - DNA, 4966 bp, synthetic construct
  source 1..4966: mol_type = other DNA
atgctttctgcaacacttccagtgtcccttacatctgcaaagggctcctccttggccttctcccgccgcatggttccttccggccaccgtctatctccggcgacactcaccggcgtttcactctcacgcgctcctctcacgttgaggtgctcttcactctcaaacaccccttcctatggtaagtgttattttggttttgctagttttgttttgagtaccccacctgaaattataggcagaatgacgaaagggtagctatcctgttcataaaaattcaatcttgttccacgtttaaataaattctacgataactgtgtaaatggtgagtggtggtttgaaagtgctttaactttgaaggcaaaaatgacaaatgggtaggtatctcgattgaaaagttttaatcttttctccgtgtttgaataagttcttcgatatcctgtgtagtaaatgagtatttgtgattttatttatttatttactaaatgatgacttaaatgtgtgtaactgtgaaggcaaaaatgacaattgggtaggtatgttgattgaaaagttttaatctttgctccatgtttgaataaatcttcaatatcctgtggtaaatgggtaggtatcctgttaaatagtgacaatttgattaattttagataagtgaaggagtctgtggctaatgttggtgcttccattcatcagcatttggttaattgcttttgtgttttcaataattataacttttttttttttggttttaatcttggacttaacatgtatgacggatactacttttgcagttgaggaaggaagaaagtttgtagaagcttcaaagaatgggaacttgattcctctctgtcagagcatcttcgctgaccaactcactcctgtccttgcttaccggattttggttaaggaagacgattgggaggctccaagctttcttttagcttcgagtgttgtgagtttgctttttggagtattgtgattttgaattttttgagttgtttgtgtctttaactctttattgaaactgaagacaagattgattgtttattgcaggggcgctatagtgttttaggagcaaacccaactatggaagttgtggcaaaagaaaataaggttacaataattgaccacgaatctgggaatttaactgaggaaattgttgatgatcctatggtgattcccagaaaaatctcagagggttggaaaccctatctcattgatgaactaccagatgcattctgtggtaagagttttatgatcataatgcccgtatttagtaaaacaactttgtgcaacgtctgtatggattactaacgtataacgtgcaacgtctgcatggacaaacaactttgtgataactgaaaatcctaagatagaagagaaaattaaatcgacttgtcgtttatgcttttataatttatagtatctgatgttgacatcttgtggttttagatgattaagattgtcacctgaatcttgctttctgcgttacttgtcgagttgtcgttacttgatgtcttatttatgttatctgtgtgcctgacgcgcagatgcttgtgtgggtgttcacttgcatgtgtgtgaaagacagagggctgtattcttgacgtgttttttcatctaattaacttgtttaagctgctcttctaggtggttgggcaggttatttctcatatgacactgttcgttatgtggaaaagaaaaagctaccattttcaaacgctccagaggatgacaggaaccttgctgacatacatctgggcctctatgagaatgtgattgtgtttgaccatgtagaaaaggtacctgtttttctatgcttcacaagtactgtatcaatgttggcatctagtttggtgtttctcacaagacatttttttgtttctaatgttgacatgtagctcactatttctaatttgcactgtagtatatcctcttatcattttaagaaaaactcaattcagattgcttcataaacaaaatgttatgatttcatttctttcctattgtttttaattggatttttgttcattgaatgaggaacaaaaaatcttttcaatgttcatgtacatgctgttttgacattattggatatataatgatctaattattatttgaagagtagaaatcatgaaatgaccaattactatttaattgcattaatatggattatattcaggattcattcatagcttcaatatttcatgttcactcgtattctgcataacagaaagcatatgtgattctttgggtgagggttgatcggtactcctcggctgagagtgcttataaggatggaatggaaagattagaaaaattagtggccaaattacaagatggccaaccgtaagtcatctattaaccgtttctctctttaatgatgtacctgttatgattgaatcaaaattaatttaaagcatgtgtttcctagcccaaggctggctccaggttctgtggatttacatactcatcattttggtccatctttaaagaagtcaagcatgacaagtgaagcatacaaagaggcagtccttcaggcaaaagaacatattaaagcaggggatattttccagattgtattaagtcagagattcgaacgaagaacatttgctgatccttttgaaatttatagagcattgagagttgttaacccaagtccttatatggcctatttgcaggtttatttctgcgtaacatctgaaacttcttccttcattcaagaaagttttatggttcagctctttcatgttctatgattatgtatttcctaaacaggctaggggatgtattctggttgcttcaagtccagagattcttacacgtgtaaagaaggtaggatttgtacatatattagatttttaaattaaattatacttatacttcttatttggtgactgggatatttgtcataaatcataaataaaaaatatattagactttgttaaattagtctattatttattttaaaacagatagttattatgattttgtcattaacagaataagattatgaaccgtccattggctgggacagctagaagggggaaaacacctgaagaagatgcaaggtttgaagcaatattgctgagagatgaaaagcagtgtgcagagcatgtcatgttggttgatttgggacgcaatgatgttggaaaggtttgttataaatattcaatataatggatactcctatttgtttttttcctgttcaaggtgtcttgaagcaatagcttggtcaattatattgttcatttaaagaaaatactgcctctcttatttcttatattatatttactctataacctcttcaattggagttgacgttttgaacacccacctttcttgtgttaatcccacaagcttctcatccattctcaattcatgatcaagacatcaaaatagaaaatcttgcattgggtttagggataagtaagcttgctttgatgacttccatcatgtcaatgctacactttacttctgtgttacacagctataccccttcccttgccccattgagaaattgaactgactaatactaagttaaaggattaagaaactcaataacactattcttacacaaatggaatcaggccttcttttctttgcacattattcaaagttacatctatcaatatgagtgtttttgtgaaagcaataaaagcaatgcaacggagaagcaacctccatgttgctttggtgtttttgctgggaaagctaaatttctccattgaacatggtttggatgtgttttcaaacacactatatagctaataattggagttcaacaatgctttcattaactgtggttgtcagtccattatctgaacttgtaagggtgttcggtgaaagccaatctgcagttagttatctggttgtgttagaagcagtaggtacatatgtatcttgttaactgctgctttgtggatttgctgtaattaagcgttcttcatttctttgtaacaaatagatatgataatacctcattttgttgtatatcatgatgtagaagaaagtaatttattctgactttttgagaaaatggtttatatttggtattgtgatgattctcgtagcaggagtttctcttttgtaggttgcaaaaagtggttctgtcaaagttgaaaagcttatgaatgttgaacgatattcccatgtcatgcacataagttcaacggtgagaatattttcttgatatcaagtgtgttggtttttcacaaaagatttcttgtaattctggttaccaacacttcccctatattattaaattgatgctgccatggttcctctgtcccaaaaaattatttctctatccaattaagtcagaacactgggtattatttcattgcatttttctgtttaaacaaaaaatgttgcttatttattgtaggttactggagagttgcaagagcatttgactagctgggatgccctgcgagctgcattgcccgttggaactgtcagtggagcaccaaaggtttgtaattttctcgacttctttttagtcaactacgaatgagaaaacgtttttgttttcattttctgttttttacttttaattacaaaactgtttccttacttccaatctatttcctgttttgaaatatgtgttcaaaactttccaccttgattcattcttatgtggatgcaggtgaaggcgatggagttgattgatgagctggaggtgacaaggagggggccttacagtggaggatttggatacatctctttctctggtgagatggacattgctcttgctctcaggacaatggtatttccgagcggaaccaggtatgatacaatgtactcatacaaagacgtcgaccaacgccgcgagtggattgcttaccttcaagccggagctggtatagttgctgacagtgtccctgatgatgagcaccaagagtgtcaaaacaaagctgctggtcttgctcgtgccattgatttggctgagtccgcttttgttgataaatga

SEQ ID NO: 6 - protein, 587 aa, synthetic construct
MLSATLPVSLTSAKGSSLAFSRRMVPSGHRLSPATLTGVSLSRAPLTLRCSSLSNTPSYVEEGRKFVEASKNGNLIPLCQSIFADQLTPVLAYRILVKEDDWEAPSFLLESAEPHASSVGRYSVLGANPTMEVVAKENKVTIIDHESGNLTEEIVDDPMVIPRKISEGWKPYLIDELPDAFCGGWAGYFSYDTVRYVEKKKLPFSNAPEDDRNLADIHLGLYENVIVFDHVEKKAYVILWVRVDRYSSAESAYKDGMERLEKLVAKLQDGQPPRLAPGSVDLHTHHFGPSLKKSSMTSEAYKEAVLQAKEHIKAGDIFQIVLSQRFERRTFADPFEIYRALRVVNPSPYMAYLQARGCILVASSPEILTRVKKNKIMNRPLAGTARRGKTPEEDARFEAILLRDEKQCAEHVMLVDLGRNDVGKVAKSGSVKVEKLMNVERYSHVMHISSTVTGELQEHLTSWDALRAALPVGTVSGAPKVKAMELIDELEVTRRGPYSGGFGYISFSGEMDIALALRTMVFPSGTRYDTMYSYKDVDQRREWIAYLQAGAGIVADSVPDDEHQECQNKAAGLARAIDLAESAFVDK

SEQ ID NO: 7 - protein, 585 aa, synthetic construct
MLSATLPVSLTSAKGSSLAFSRRMVPSGHRLSPATLTGVSLSRAPLTLRCSSLSNTPSYVEEGRKFVEASKNGNLIPLCQSIFADQLTPVLAYRILVKEDDWEAPSFLLESADASSVGRYSVLGANPTMEVVAKENKVTIIDHESGNLTEEIVDDPMVIPRKISEGWKPYLIDELPDAFCGGWAGYFSYDTVRYVEKKKLPFSNAPEDDRNLADIHLGLYENVIVFDHVEKKAYVILWVRVDRYSSAESAYKDGMERLEKLVAKLQDGQPPRLAPGSVDLHTHHFGPSLKKSSMTSEAYKEAVLQAKEHIKAGDIFQIVLSQRFERRTFADPFEIYRALRVVNPSPYMAYLQARGCILVASSPEILTRVKKNKIMNRPLAGTARRGKTPEEDARFEAILLRDEKQCAEHVMLVDLGRNDVGKVAKSGSVKVEKLMNVERYSHVMHISSTVTGELQEHLTSWDALRAALPVGTVSGAPKVKAMELIDELEVTRRGPYSGGFGYISFSGEMDIALALRTMVFPSGTRYDTMYSYKDVDQRREWIAYLQAGAGIVADSVPDDEHQECQNKAAGLARAIDLAESAFVDK

SEQ ID NO: 8 - protein, 581 aa, synthetic construct
MLSATLPVSLTSAKGSSLAFSRRMVPSGHRLSPATLTGVSLSRAPLTLRCSSLSNTPSYVEEGRKFVEASKNGNLIPLCQSIFADQLTPVLAYRILVKEDDWEAPSFLLASSVGRYSVLGANPTMEVVAKENKVTIIDHESGNLTEEIVDDPMVIPRKISEGWKPYLIDELPDAFCGGWAGYFSYDTVRYVEKKKLPFSNAPEDDRNLADIHLGLYENVIVFDHVEKKAYVILWVRVDRYSSAESAYKDGMERLEKLVAKLQDGQPPRLAPGSVDLHTHHFGPSLKKSSMTSEAYKEAVLQAKEHIKAGDIFQIVLSQRFERRTFADPFEIYRALRVVNPSPYMAYLQARGCILVASSPEILTRVKKNKIMNRPLAGTARRGKTPEEDARFEAILLRDEKQCAEHVMLVDLGRNDVGKVAKSGSVKVEKLMNVERYSHVMHISSTVTGELQEHLTSWDALRAALPVGTVSGAPKVKAMELIDELEVTRRGPYSGGFGYISFSGEMDIALALRTMVFPSGTRYDTMYSYKDVDQRREWIAYLQAGAGIVADSVPDDEHQECQNKAAGLARAIDLAESAFVDK

SEQ ID NO: 9 - DNA, 4293 bp, Glycine max
  source 1..4293: mol_type = genomic DNA
atgtcgtcgttgataacagatttgctccgtcaaaccggcggcaccgccgtcatcgacggcggtctggcgacggagctggagcgccatggcgccgacctcaatgatcctctttggagcgccaagtgcctcttttccttccctcacctcattcgccaagtacaatccgtttcgaatctaacgcaccgtttcaactctcaaatttttgttctatttttccattattaaataaatctctgtgatttcatttcatcagtgttaattgatttcacgaaccagatttttttgcttatatcattgttaagcagttcttgcaatgttactatttttagcttaattgaatcatgtgtttttgtctttttttccttttttaattttttgcaattgaaaattaaagtaatgattgaatgactaaatggagcaggtgcaccttgattacctggaaaatggtgcagacattataatcacagcatcttaccaagtgagttagttggtttggttgttgagcagtgtcttatttctttgttaatttctttctaatgctgaagtcgaggtacttgtgttgtttgtgcacaggccaccattcaagggtttaaagccaaaggctattctgatgaagagagtgaagccttgctcagaagcagtgttgaaattgcacgggaggcacgcgaagtttactataaaaattgtgctggatgtcgttcgggtgatggggatgatgatggtagaatcctcaaacaacggcctatcttggttgctgcatcagtagggagctatggggcttatttggccgacgggtcagagtacaggtgaaatgaatcaaacgattaagatttagtatctagacttcgtttggataaacttctttataagcactagtataggaaaataatataaggtagtaaaacgaattgaacttctctcctatgctaaaatcaacttatgtacttaacttttgtggaagcgttagcatctaatttctctaaaagctaaagtgtttcagttgattttagtttattgagagaggttcagttcatttaatctttttatattcttttcttatataagttcttagggggaaatttatctaaactgagtcatagcattgtttgtgatttttgttttcttgtatctattatgtagcccatttattaacaaacaatcaaggtgatattcatgatcattataagttgtgtttcccaggtcgtgtatttagctttgtattggttattttggtacaaatctttcttgttcttaaagggaatggtatcagaaagttgtatgaaatgaacttctagttccatcttgtgcttacatatttgagcttttttctgcataggatcattgacatttttagaaaggttggggtttgataatgtttgcttctgttctcagcactgatagaaattatatattttttagtgtcacgtttcttgatattttgtttctaacagtggggattatggtgatgctatcacggtggaaactcttaaagattttcatcggagaagagttcaaattttagcagattcaggtgctgacctgcttgcatttgaaacagttcccaataagcttgaagctgaggtatcctacagctttggacagccaaatgctaaaatttactcacatggttcttttttatccctatctgtcatccatctcttaaaaattattgaagcataatcttttttcaaactttacccttaatatttatgagtgagagaagatcaatcaatattttaatattttgaattttctaatgaagggtaattcagtcaaatgaacttgttttgcttataattgaggctatctaatgacattcttatttcttgtgcaataaccttaaagtgtggataatgaatggtaatcaaattcttgatgattgaagaaattctgtgatatttgtataattcattttggttgatgtgctttttttctatgttaccatgaaatgtgaatcacaaacttttgatggatgttttctttgagtgaagaagttttcaacaaaaatttggcccaaattttgccttgcttccctagaccacaggaaaccaagaaagcattaaatttctattctggagtttccattgcttttgtgaaagcataaaatcactagtaaagtaactataatgagtaactcattaaagcatatataatcaattaaaatcccagaaaaagtacaaaataatagttatctaaagctaaatattggtcttggacaattaaactttgcaagtcttcacttgcaatgttcattttttgtcttgactcctgaatttacctaactatattgactataagcaggcttatgctcagcttctggaagaagaggacataaaaattcctgcatggttttcttttaactctaaggatggagttaatgttgttagcggtgattctttaatggaatgtggctctattgctgaatcatgtaataaagttgtcgctgttggaatcaactgtactccaccaagatttattcatggtctgattgttttgcttaagaaggtaaaacttaggttctcttgtttccaatatgttgtgtgtaggctaactattgaacttatttttttacacatcataaattcatattttgtttttatcaacctctcctactcttttaggtcattattagtactgctgtttcagttctaagtgttagtattcatgctgccaagttgttttcattttgataagtcgtgtacattagggtggataataaatacacatggatgttaatctgtataggttcaaccattcaagagttgcataatattgtaaatagccttcaactatttttaattctttatttttttataaagatggcttatatgaacggaaacttctctgaataaagtacttaacctataccctgatacagttttcgcattaatgtacaactatttgtctctagaatgtaggtaatgtcattttcccgtgtttttttgtgttacttttgtgtgaggaatgtgccagtgttgataagctatcatattgttatagttatgggacttgtctttgtggaatacttatccttgattcacatatggtttcttcaggtgactacaaaaccaattgttatatatccaaacagtggggaaacttacgatgctgacctaaaggagtgggtggtaagtttatttcatgtgattgtactattacattttaaaggataggcaggcctactttgtcttaaaaattgaagaaagatctattatagaatataagtatcaaaattatcatataaaaaatgagccacttggattatggaaattattctgctttaattaaagtaattcatattctgtcaaataaaagaaagaagctgtaaaggcaaacttaattatagagtaaaagtatataggtgtgtccctatcccttctcttttccattttggtgaaatcattttatttgaactgtacaactgattcagattgttgtgtcatgtgtgatttatcatttaaaatagaaacttgctcagaagtaggagtcttagtgtaagtggtagcttagtactggtatggaatgacagatttcacatccttttattaataatcgtatacaagtacatatgaagattttaaggaaagacttgaatagttttttagcccctataatatatacagggttgttttctttttgtcctcttaattttttttttcctgttttggtccttataaaatgtttttgtttcatttggatccctgtcctagttaagtgatgacatggttaatagagattagaaaatagccaaatgtgcactcatgtgttggacatggttaagagagattagtgattatttaatcatgttccgcctgtgcaattttctatatttcttgtaacacaatagcaaacaatgcatgtaacatgatatcataagaaattaatggaaccccacatgaacatgaattaactccttaagttatgtatttgttttatctagtttattgtatttttcaagttatgaacttatggtttgttaaagttgattagtacttcatatggtacacattcttatctttgagagaaaccacataaagcatggagatagtttcttagagattcaatcattttaaagaaaatattttgggatgtttcttgaattatgtatacagtcacactgatattatgctgttgttattgcagcaaaatactggtgttacagatgaagattttatctcatatgtaaataaatggtgtgagttaggagcttcccttgtaggtggctgttgcagaacgactccggatactattaggaagatatacaggaccctgtctagcagtcaatcaatctaa

SEQ ID NO: 10 - protein, 333 aa, Glycine max
MSSLITDLLRQTGGTAVIDGGLATELERHGADLNDPLWSAKCLFSFPHLIRQVHLDYLENGADIIITASYQATIQGFKAKGYSDEESEALLRSSVEIAREAREVYYKNCAGCRSGDGDDDGRILKQRPILVAASVGSYGAYLADGSEYSGDYGDAITVETLKDFHRRRVQILADSGADLLAFETVPNKLEAEAYAQLLEEEDIKIPAWFSFNSKDGVNVVSGDSLMECGSIAESCNKVVAVGINCTPPRFIHGLIVLLKKVTTKPIVIYPNSGETYDADLKEWVQNTGVTDEDFISYVNKWCELGASLVGGCCRTTPDTIRKIYRTLSSSQSI

SEQ ID NO: 11 - DNA, 4290 bp, synthetic construct
  source 1..4290: mol_type = other DNA
atgtcgtcgttgataacagatttgctccgtcaaaccggcggcaccgccgtcatcgacggcggtctggcgacggagctggagcgccatggcgccgacctcaatgatcctctttggagcgccaagtgcctcttttccttccctcacctcattcgccaagtacaatccgtttcgaatctaacgcaccgtttcaactctcaaatttttgttctatttttccattattaaataaatctctgtgatttcatttcatcagtgttaattgatttcacgaaccagatttttttgcttatatcattgttaagcagttcttgcaatgttactatttttagcttaattgaatcatgtgtttttgtctttttttccttttttaattttttgcaattgaaaattaaagtaatgattgaatgactaaatggagcaggtgcaccttgattacctggaaaatggtgcagacattataatcacagcatcttaccaagtgagttagttggtttggttgttgagcagtgtcttatttctttgttaatttctttctaatgctgaagtcgaggtacttgtgttgtttgtgcacaggccaccattcaagggtttaaagccaaaggctattctgatgaagagagtgaagccttgctcagaagcagtgttgaaattgcacgggaggcacgcgaagtttactataaaaattgtgctggatgtcgttcgggtgatggggatgatggtagaatcctcaaacaacggcctatcttggttgctgcatcagtagggagctatggggcttatttggccgacgggtcagagtacaggtgaaatgaatcaaacgattaagatttagtatctagacttcgtttggataaacttctttataagcactagtataggaaaataatataaggtagtaaaacgaattgaacttctctcctatgctaaaatcaacttatgtacttaacttttgtggaagcgttagcatctaatttctctaaaagctaaagtgtttcagttgattttagtttattgagagaggttcagttcatttaatctttttatattcttttcttatataagttcttagggggaaatttatctaaactgagtcatagcattgtttgtgatttttgttttcttgtatctattatgtagcccatttattaacaaacaatcaaggtgatattcatgatcattataagttgtgtttcccaggtcgtgtatttagctttgtattggttattttggtacaaatctttcttgttcttaaagggaatggtatcagaaagttgtatgaaatgaacttctagttccatcttgtgcttacatatttgagcttttttctgcataggatcattgacatttttagaaaggttggggtttgataatgtttgcttctgttctcagcactgatagaaattatatattttttagtgtcacgtttcttgatattttgtttctaacagtggggattatggtgatgctatcacggtggaaactcttaaagattttcatcggagaagagttcaaattttagcagattcaggtgctgacctgcttgcatttgaaacagttcccaataagcttgaagctgaggtatcctacagctttggacagccaaatgctaaaatttactcacatggttcttttttatccctatctgtcatccatctcttaaaaattattgaagcataatcttttttcaaactttacccttaatatttatgagtgagagaagatcaatcaatattttaatattttgaattttctaatgaagggtaattcagtcaaatgaacttgttttgcttataattgaggctatctaatgacattcttatttcttgtgcaataaccttaaagtgtggataatgaatggtaatcaaattcttgatgattgaagaaattctgtgatatttgtataattcattttggttgatgtgctttttttctatgttaccatgaaatgtgaatcacaaacttttgatggatgttttctttgagtgaagaagttttcaacaaaaatttggcccaaattttgccttgcttccctagaccacaggaaaccaagaaagcattaaatttctattctggagtttccattgcttttgtgaaagcataaaatcactagtaaagtaactataatgagtaactcattaaagcatatataatcaattaaaatcccagaaaaagtacaaaataatagttatctaaagctaaatattggtcttggacaattaaactttgcaagtcttcacttgcaatgttcattttttgtcttgactcctgaatttacctaactatattgactataagcaggcttatgctcagcttctggaagaagaggacataaaaattcctgcatggttttcttttaactctaaggatggagttaatgttgttagcggtgattctttaatggaatgtggctctattgctgaatcatgtaataaagttgtcgctgttggaatcaactgtactccaccaagatttattcatggtctgattgttttgcttaagaaggtaaaacttaggttctcttgtttccaatatgttgtgtgtaggctaactattgaacttatttttttacacatcataaattcatattttgtttttatcaacctctcctactcttttaggtcattattagtactgctgtttcagttctaagtgttagtattcatgctgccaagttgttttcattttgataagtcgtgtacattagggtggataataaatacacatggatgttaatctgtataggttcaaccattcaagagttgcataatattgtaaatagccttcaactatttttaattctttatttttttataaagatggcttatatgaacggaaacttctctgaataaagtacttaacctataccctgatacagttttcgcattaatgtacaactatttgtctctagaatgtaggtaatgtcattttcccgtgtttttttgtgttacttttgtgtgaggaatgtgccagtgttgataagctatcatattgttatagttatgggacttgtctttgtggaatacttatccttgattcacatatggtttcttcaggtgactacaaaaccaattgttatatatccaaacagtggggaaacttacgatgctgacctaaaggagtgggtggtaagtttatttcatgtgattgtactattacattttaaaggataggcaggcctactttgtcttaaaaattgaagaaagatctattatagaatataagtatcaaaattatcatataaaaaatgagccacttggattatggaaattattctgctttaattaaagtaattcatattctgtcaaataaaagaaagaagctgtaaaggcaaacttaattatagagtaaaagtatataggtgtgtccctatcccttctcttttccattttggtgaaatcattttatttgaactgtacaactgattcagattgttgtgtcatgtgtgatttatcatttaaaatagaaacttgctcagaagtaggagtcttagtgtaagtggtagcttagtactggtatggaatgacagatttcacatccttttattaataatcgtatacaagtacatatgaagattttaaggaaagacttgaatagttttttagcccctataatatatacagggttgttttctttttgtcctcttaattttttttttcctgttttggtccttataaaatgtttttgtttcatttggatccctgtcctagttaagtgatgacatggttaatagagattagaaaatagccaaatgtgcactcatgtgttggacatggttaagagagattagtgattatttaatcatgttccgcctgtgcaattttctatatttcttgtaacacaatagcaaacaatgcatgtaacatgatatcataagaaattaatggaaccccacatgaacatgaattaactccttaagttatgtatttgttttatctagtttattgtatttttcaagttatgaacttatggtttgttaaagttgattagtacttcatatggtacacattcttatctttgagagaaaccacataaagcatggagatagtttcttagagattcaatcattttaaagaaaatattttgggatgtttcttgaattatgtatacagtcacactgatattatgctgttgttattgcagcaaaatactggtgttacagatgaagattttatctcatatgtaaataaatggtgtgagttaggagcttcccttgtaggtggctgttgcagaacgactccggatactattaggaagatatacaggaccctgtctagcagtcaatcaatctaa

SEQ ID NO: 12 - DNA, 4227 bp, synthetic construct
  source 1..4227: mol_type = other DNA
atgtcgtcgttgataacagatttgctccgtcaaaccggcggcaccgccgtcatcgacggcggtctggcgacggagctggagcgccatggcgccgacctcaatgatcctctttggagcgccaagtgcctcttttccttccctcacctcattcgccaagtacaatccgtttcgaatctaacgcaccgtttcaactctcaaatttttgttctatttttccattattaaataaatctctgtgatttcatttcatcagtgttaattgatttcacgaaccagatttttttgcttatatcattgttaagcagttcttgcaatgttactatttttagcttaattgaatcatgtgtttttgtctttttttccttttttaattttttgcaattgaaaattaaagtaatgattgaatgactaaatggagcaggtgcaccttgattacctggaaaatggtgcagacattataatcacagcatcttaccaagtgagttagttggtttggttgttgagcagtgtcttatttctttgttaatttctttctaatgctgaagtcgaggtacttgtgttgtttgtgcacaggccaccattcaagggtttaaagccaaaggctattctgatgaagagagtgaagccttgctcagaagcagtgttgaaattgcacgggaggcacgcgaagtttactataaaaattgtgctggatcagtagggagctatggggcttatttggccgacgggtcagagtacaggtgaaatgaatcaaacgattaagatttagtatctagacttcgtttggataaacttctttataagcactagtataggaaaataatataaggtagtaaaacgaattgaacttctctcctatgctaaaatcaacttatgtacttaacttttgtggaagcgttagcatctaatttctctaaaagctaaagtgtttcagttgattttagtttattgagagaggttcagttcatttaatctttttatattcttttcttatataagttcttagggggaaatttatctaaactgagtcatagcattgtttgtgatttttgttttcttgtatctattatgtagcccatttattaacaaacaatcaaggtgatattcatgatcattataagttgtgtttcccaggtcgtgtatttagctttgtattggttattttggtacaaatctttcttgttcttaaagggaatggtatcagaaagttgtatgaaatgaacttctagttccatcttgtgcttacatatttgagcttttttctgcataggatcattgacatttttagaaaggttggggtttgataatgtttgcttctgttctcagcactgatagaaattatatattttttagtgtcacgtttcttgatattttgtttctaacagtggggattatggtgatgctatcacggtggaaactcttaaagattttcatcggagaagagttcaaattttagcagattcaggtgctgacctgcttgcatttgaaacagttcccaataagcttgaagctgaggtatcctacagctttggacagccaaatgctaaaatttactcacatggttcttttttatccctatctgtcatccatctcttaaaaattattgaagcataatcttttttcaaactttacccttaatatttatgagtgagagaagatcaatcaatattttaatattttgaattttctaatgaagggtaattcagtcaaatgaacttgttttgcttataattgaggctatctaatgacattcttatttcttgtgcaataaccttaaagtgtggataatgaatggtaatcaaattcttgatgattgaagaaattctgtgatatttgtataattcattttggttgatgtgctttttttctatgttaccatgaaatgtgaatcacaaacttttgatggatgttttctttgagtgaagaagttttcaacaaaaatttggcccaaattttgccttgcttccctagaccacaggaaaccaagaaagcattaaatttctattctggagtttccattgcttttgtgaaagcataaaatcactagtaaagtaactataatgagtaactcattaaagcatatataatcaattaaaatcccagaaaaagtacaaaataatagttatctaaagctaaatattggtcttggacaattaaactttgcaagtcttcacttgcaatgttcattttttgtcttgactcctgaatttacctaactatattgactataagcaggcttatgctcagcttctggaagaagaggacataaaaattcctgcatggttttcttttaactctaaggatggagttaatgttgttagcggtgattctttaatggaatgtggctctattgctgaatcatgtaataaagttgtcgctgttggaatcaactgtactccaccaagatttattcatggtctgattgttttgcttaagaaggtaaaacttaggttctcttgtttccaatatgttgtgtgtaggctaactattgaacttatttttttacacatcataaattcatattttgtttttatcaacctctcctactcttttaggtcattattagtactgctgtttcagttctaagtgttagtattcatgctgccaagttgttttcattttgataagtcgtgtacattagggtggataataaatacacatggatgttaatctgtataggttcaaccattcaagagttgcataatattgtaaatagccttcaactatttttaattctttatttttttataaagatggcttatatgaacggaaacttctctgaataaagtacttaacctataccctgatacagttttcgcattaatgtacaactatttgtctctagaatgtaggtaatgtcattttcccgtgtttttttgtgttacttttgtgtgaggaatgtgccagtgttgataagctatcatattgttatagttatgggacttgtctttgtggaatacttatccttgattcacatatggtttcttcaggtgactacaaaaccaattgttatatatccaaacagtggggaaacttacgatgctgacctaaaggagtgggtggtaagtttatttcatgtgattgtactattacattttaaaggataggcaggcctactttgtcttaaaaattgaagaaagatctattatagaatataagtatcaaaattatcatataaaaaatgagccacttggattatggaaattattctgctttaattaaagtaattcatattctgtcaaataaaagaaagaagctgtaaaggcaaacttaattatagagtaaaagtatataggtgtgtccctatcccttctcttttccattttggtgaaatcattttatttgaactgtacaactgattcagattgttgtgtcatgtgtgatttatcatttaaaatagaaacttgctcagaagtaggagtcttagtgtaagtggtagcttagtactggtatggaatgacagatttcacatccttttattaataatcgtatacaagtacatatgaagattttaaggaaagacttgaatagttttttagcccctataatatatacagggttgttttctttttgtcctcttaattttttttttcctgttttggtccttataaaatgtttttgtttcatttggatccctgtcctagttaagtgatgacatggttaatagagattagaaaatagccaaatgtgcactcatgtgttggacatggttaagagagattagtgattatttaatcatgttccgcctgtgcaattttctatatttcttgtaacacaatagcaaacaatgcatgtaacatgatatcataagaaattaatggaaccccacatgaacatgaattaactccttaagttatgtatttgttttatctagtttattgtatttttcaagttatgaacttatggtttgttaaagttgattagtacttcatatggtacacattcttatctttgagagaaaccacataaagcatggagatagtttcttagagattcaatcattttaaagaaaatattttgggatgtttcttgaattatgtatacagtcacactgatattatgctgttgttattgcagcaaaatactggtgttacagatgaagattttatctcatatgtaaataaatggtgtgagttaggagcttcccttgtaggtggctgttgcagaacgactccggatactattaggaagatatacaggaccctgtctagcagtcaatcaatctaa

SEQ ID NO: 13 - DNA, 4646 bp, Glycine max
  source 1..4646: mol_type = genomic DNA
atggggttagaagggaaggaaacgccgtcgtttatgagggattttctcgataagtgtggtggctgcgccgttattgacggtggttttgccactgaacttgaaaggcatggggcggacctcaatgacgaactctggagtgccaaatgccttattagctccccacatcttgtccgaagggtactttttcttcttctttatcatttaattttgctattggttttctttttaagaatgttatttagagtaatactctcaactctcaactttcttttagagttaatgcatgctagtttatagtttatcatatgggtgtagcttaattgataacactcggtttgtgaggaaaacacacgcagaatttacggtggaacacctggatttgatcctgcataatggatatttggggggtcctccctaatgactgaggtcggaaaaaaaagttaatgggttaccatagccactagaaactagaaactgcaaaattaatttgaattaatagcaatattctatgtaacaatttcttttttctttttaagtgaatgacggagatgaattgtgataaaattaggcattattggattagttttaaaaaactgggaaaaaagtatgatttgtcttttgtttgaaagaagggaaaaggtatgatagttacttataactacagtatggaattatatttatttatctaattttaaattttaattctaagataatgatgtgtataaaaacaataatttgcgttttttttttaaatattcgatatattcaaagcatagtcataataaataatttttatttatttaacttgtgttttaaaatccacatgcactaacaaattatctttaagttattatatttatatacttaattattattatttttttcattttgatctttttcttcatttttcattccattatttataacctgtataaacttttctttctttagtatttgctctttctgtcttcccttcttccaccaatacatcccaaatttgggatatacgttgtttttctcccagttcttttataaagggaggagagacaaacttagtgctttaaaaatacacgtaacaaattctttgtcaatattatgtatgatagcaccgatagacctacttacgtcaacatgaaacagcaaagaaaattatgtaagagaaaaaagaccaagaacgaatttacaacgcacgcgtagcagattatattgtccacgtgttattgtttaatgggtcctggtgttacgtgtaaggcatttagggtgggcaaatgcatgtttttcttagctaattgccctgccaataagaagaggtgttcgcagtaagaaagataaactttaatacatgctcaaagtaaaattcttagttaatgatttatttttaatttaaatttaactcaacattttatatttatttataagatattatgattatatatttaatttcacactaagtatcgtgtttttagaatatagaataatctttttaagagacttaaaaattaaaaggttaactgttctaaaaaaatcattaaactaaaggagactaagaagggaaaattgaaatcatgaaagcaaattaaagaaacttgtctattgtatataactttttttgatacatgtctatattatataatattgaccaatttatttgctttattcttgataagataaactagactttcttgtaaaagataaccattgctttaattaggaggaccttatctcatggatgaggttgacatgtttgtgtgtatcatagaaatgatagacagaaatccagaattttaaaggacctatctcatgaatgaggttgacatgtttgtgtgtatcatagaaataaattcagaatttatttataaagatgagtttcatattacaaggagttttttttatatagaattgagaaaggaaacacacacaaactaagcagtagttcagctatttatactgattttttacaaataaacaactcactaatattagtaatttgttacaattgttttaactacaagcttagtttgttagaactattttaattaccaacttaatttgttacttatgtgaaccaacctatcaacaatttgcatatataggatatgattacgaaatttcagacgcattgtacactgtttataaccaaataacccaacaaggtttgatgaaagaaaaggaggagtacaaacaaaagaccaaagttgccaatcccaactgttgttgcctttgtggatcttggtgtgttaatcttatatataatatacacattcactttttaaattttttttattagtgcttaataattaatatccgattgatggtttattagtacaatttttaataattaatggtttattagtataatttttatttaatacaaaataaattattagtataggaatttccattaattctttctaggttggtcgagtatagaaatttccattaactatattctgaattttccttccctttctaaaagatctgcagtttcacacgagtgatcaaaggaatgggaaaaaaatgtaatagaaaattaccttagtttagtatttaatttttgaacaggcaacaactgttcatttcatgaaactcattttgcttaacgtggacaggttcacctagattacctcgatgcaggagcaaacataatattaacagcatcttatcaggtaattatcatattaattttttttttcatccctacaactctacattttaattttgccgtctttttggggttggggtgcaggccactattcaaggttttgaggccaaagggttctctagagaagaaggtgaaactatgcttagaagaagtgtggagattgcacgtgaggcacgagaaatttattatgataggtgcaccaaagattcttctgactttatgagagatgaaagatataggaaacgtcccattttaattgcagcttctgtgggaagctatggagcgtatttggctgatggctctgaatatgtgtgagtgaacaaaaccaattatgtcaaaatagtcattaaagttggacttatgttgatttcaattaatattcactgttttgttactttttagtttgtagcataaatttttaacaactagttctgaattgcaaatataatttactaattgtatttgagtttaagatgaaaattttcatgattgaagtcaaaactgtacttccaaaataaagcaatgttgcagcaatatatatgacttaagtctacattgatttttctctcttcacagtggggactatggtgatgcagttactgtccagacactgaaagattttcacagggaaagagtaaagattcttgttgaggctggtgctgacttaatagcctttgaaacaattccaaataagctggaggcacaggtatttactaactaacaaacagactcacttatttgttacttgctttttatgtctgaaacagtaagaatctgtaatagaaatgttcaaaatgcagtgtcaattaccatttactaataccatagaaaattggaaattaccattgcatttttgtctagtttctccttgattttgagcaatcttattaattttcgttacaatttgataaataggcttatgctgaacttctcgaggaagaaggcatagaaactcctgcgtggttttcttttagttgtaaggatgaaagcaatgtggttagtggtgactctatctttgaatgcgcttcaatagctgattcatgcagacaagttgttgcggttggagttaattgtactgctcctagatttattcatggattgatttcatttatcaagaaggtgcaactttcaaataatactctgctctacactatcaaaatgtgctaattggcaatattgttttgaataacttgtgagttggccttctagttgattgtatactgtgcatgaaatgttctttaactagtgtctttaaggtactcgttgctagaagaccttataaactattctcaagtgagaaatgctaataacactaatttgtccgataacagctcactttatgacagaatttaacactccgtttttaaatagcaggcaacaagtaaaccagtacttgtatatcccaacagtggggagacttatatcgctgagagcaaccaatgggtggtgagttctgcttctctctttttacatggcctcagcttgtttttatgttcatgtttaaccaacttcaaatctaattccagttataataaatgatacttcctcatcaatttaaatgtctgaacctcatttttgcatgttttcaagtccttgttacgaatcttttcattgacattctataatttgcaacgtgaatttcgaaatataatctaaatgaagttactaaaaagcaaatcaacatgcacacattctgcatacactgccactttagtggtgtggacagaacactttttttttgttaaaccacaatgtgctataagaattcgtatatataattctagtttagtatcatcaaattgataacttaaaatttgtcttatagaaatcaagtggggcagcagagcatgattttgtctcctacataggcaagtggcgtgatgctggggcttccctttttggtggctgctgcaggactactcctaatactataagaggcatagcagaggcaacatatgggaaacttaaagacaaatgtatataa

SEQ ID NO: 14 - protein, 342 aa, Glycine max
MGLEGKETPSFMRDFLDKCGGCAVIDGGFATELERHGADLNDELWSAKCLISSPHLVRRVHLDYLDAGANIILTASYQATIQGFEAKGFSREEGETMLRRSVEIAREAREIYYDRCTKDSSDFMRDERYRKRPILIAASVGSYGAYLADGSEYVGDYGDAVTVQTLKDFHRERVKILVEAGADLIAFETIPNKLEAQAYAELLEEEGIETPAWFSFSCKDESNVVSGDSIFECASIADSCRQVVAVGVNCTAPRFIHGLISFIKKQATSKPVLVYPNSGETYIAESNQWVKSSGAAEHDFVSYIGKWRDAGASLFGGCCRTTPNTIRGIAEATYGKLKDKCI

SEQ ID NO: 15 - DNA, 4644 bp, synthetic construct
  source 1..4644: mol_type = other DNA
atggggttagaagggaaggaaacgccgtcgtttatgagggattttctcgataagtgtggtggctgcgccgttattgacggtggttttgccactgaacttgaaaggcatggggcggacctcaatgacgaactctggagtgccaaatgccttattagctccccacatcttgtccgaagggtactttttcttcttctttatcatttaattttgctattggttttctttttaagaatgttatttagagtaatactctcaactctcaactttcttttagagttaatgcatgctagtttatagtttatcatatgggtgtagcttaattgataacactcggtttgtgaggaaaacacacgcagaatttacggtggaacacctggatttgatcctgcataatggatatttggggggtcctccctaatgactgaggtcggaaaaaaaagttaatgggttaccatagccactagaaactagaaactgcaaaattaatttgaattaatagcaatattctatgtaacaatttcttttttctttttaagtgaatgacggagatgaattgtgataaaattaggcattattggattagttttaaaaaactgggaaaaaagtatgatttgtcttttgtttgaaagaagggaaaaggtatgatagttacttataactacagtatggaattatatttatttatctaattttaaattttaattctaagataatgatgtgtataaaaacaataatttgcgttttttttttaaatattcgatatattcaaagcatagtcataataaataatttttatttatttaacttgtgttttaaaatccacatgcactaacaaattatctttaagttattatatttatatacttaattattattatttttttcattttgatctttttcttcatttttcattccattatttataacctgtataaacttttctttctttagtatttgctctttctgtcttcccttcttccaccaatacatcccaaatttgggatatacgttgtttttctcccagttcttttataaagggaggagagacaaacttagtgctttaaaaatacacgtaacaaattctttgtcaatattatgtatgatagcaccgatagacctacttacgtcaacatgaaacagcaaagaaaattatgtaagagaaaaaagaccaagaacgaatttacaacgcacgcgtagcagattatattgtccacgtgttattgtttaatgggtcctggtgttacgtgtaaggcatttagggtgggcaaatgcatgtttttcttagctaattgccctgccaataagaagaggtgttcgcagtaagaaagataaactttaatacatgctcaaagtaaaattcttagttaatgatttatttttaatttaaatttaactcaacattttatatttatttataagatattatgattatatatttaatttcacactaagtatcgtgtttttagaatatagaataatctttttaagagacttaaaaattaaaaggttaactgttctaaaaaaatcattaaactaaaggagactaagaagggaaaattgaaatcatgaaagcaaattaaagaaacttgtctattgtatataactttttttgatacatgtctatattatataatattgaccaatttatttgctttattcttgataagataaactagactttcttgtaaaagataaccattgctttaattaggaggaccttatctcatggatgaggttgacatgtttgtgtgtatcatagaaatgatagacagaaatccagaattttaaaggacctatctcatgaatgaggttgacatgtttgtgtgtatcatagaaataaattcagaatttatttataaagatgagtttcatattacaaggagttttttttatatagaattgagaaaggaaacacacacaaactaagcagtagttcagctatttatactgattttttacaaataaacaactcactaatattagtaatttgttacaattgttttaactacaagcttagtttgttagaactattttaattaccaacttaatttgttacttatgtgaaccaacctatcaacaatttgcatatataggatatgattacgaaatttcagacgcattgtacactgtttataaccaaataacccaacaaggtttgatgaaagaaaaggaggagtacaaacaaaagaccaaagttgccaatcccaactgttgttgcctttgtggatcttggtgtgttaatcttatatataatatacacattcactttttaaattttttttattagtgcttaataattaatatccgattgatggtttattagtacaatttttaataattaatggtttattagtataatttttatttaatacaaaataaattattagtataggaatttccattaattctttctaggttggtcgagtatagaaatttccattaactatattctgaattttccttccctttctaaaagatctgcagtttcacacgagtgatcaaaggaatgggaaaaaaatgtaatagaaaattaccttagtttagtatttaatttttgaacaggcaacaactgttcatttcatgaaactcattttgcttaacgtggacaggttcacctagattacctcgatgcaggagcaaacataatattaacagcatcttatcaggtaattatcatattaattttttttttcatccctacaactctacattttaattttgccgtctttttggggttggggtgcaggccactattcaaggttttgaggccaaagggttctctagaagaaggtgaaactatgcttagaagaagtgtggagattgcacgtgaggcacgagaaatttattatgataggtgcaccaaagattcttctgactttatgagagatgaaagatataggaaacgtcccattttaattgcagcttctgtgggaagctatggagcgtatttggctgatggctctgaatatgtgtgagtgaacaaaaccaattatgtcaaaatagtcattaaagttggacttatgttgatttcaattaatattcactgttttgttactttttagtttgtagcataaatttttaacaactagttctgaattgcaaatataatttactaattgtatttgagtttaagatgaaaattttcatgattgaagtcaaaactgtacttccaaaataaagcaatgttgcagcaatatatatgacttaagtctacattgatttttctctcttcacagtggggactatggtgatgcagttactgtccagacactgaaagattttcacagggaaagagtaaagattcttgttgaggctggtgctgacttaatagcctttgaaacaattccaaataagctggaggcacaggtatttactaactaacaaacagactcacttatttgttacttgctttttatgtctgaaacagtaagaatctgtaatagaaatgttcaaaatgcagtgtcaattaccatttactaataccatagaaaattggaaattaccattgcatttttgtctagtttctccttgattttgagcaatcttattaattttcgttacaatttgataaataggcttatgctgaacttctcgaggaagaaggcatagaaactcctgcgtggttttcttttagttgtaaggatgaaagcaatgtggttagtggtgactctatctttgaatgcgcttcaatagctgattcatgcagacaagttgttgcggttggagttaattgtactgctcctagatttattcatggattgatttcatttatcaagaaggtgcaactttcaaataatactctgctctacactatcaaaatgtgctaattggcaatattgttttgaataacttgtgagttggccttctagttgattgtatactgtgcatgaaatgttctttaactagtgtctttaaggtactcgttgctagaagaccttataaactattctcaagtgagaaatgctaataacactaatttgtccgataacagctcactttatgacagaatttaacactccgtttttaaatagcaggcaacaagtaaaccagtacttgtatatcccaacagtggggagacttatatcgctgagagcaaccaatgggtggtgagttctgcttctctctttttacatggcctcagcttgtttttatgttcatgtttaaccaacttcaaatctaattccagttataataaatgatacttcctcatcaatttaaatgtctgaacctcatttttgcatgttttcaagtccttgttacgaatcttttcattgacattctataatttgcaacgtgaatttcgaaatataatctaaatgaagttactaaaaagcaaatcaacatgcacacattctgcatacactgccactttagtggtgtggacagaacactttttttttgttaaaccacaatgtgctataagaattcgtatatataattctagtttagtatcatcaaattgataacttaaaatttgtcttatagaaatcaagtggggcagcagagcatgattttgtctcctacataggcaagtggcgtgatgctggggcttccctttttggtggctgctgcaggactactcctaatactataagaggcatagcagaggcaacatatgggaaacttaaagacaaatgtatataa

SEQ ID NO: 16 - DNA, 4633 bp, synthetic construct
  source 1..4633: mol_type = other DNA
atggggttagaagggaaggaaacgccgtcgtttatgagggattttctcgataagtgtggtggctgcgccgttattgacggtggttttgccactgaacttgaaaggcatggggcggacctcaatgacgaactctggagtgccaaatgccttattagctccccacatcttgtccgaagggtactttttcttcttctttatcatttaattttgctattggttttctttttaagaatgttatttagagtaatactctcaactctcaactttcttttagagttaatgcatgctagtttatagtttatcatatgggtgtagcttaattgataacactcggtttgtgaggaaaacacacgcagaatttacggtggaacacctggatttgatcctgcataatggatatttggggggtcctccctaatgactgaggtcggaaaaaaaagttaatgggttaccatagccactagaaactagaaactgcaaaattaatttgaattaatagcaatattctatgtaacaatttcttttttctttttaagtgaatgacggagatgaattgtgataaaattaggcattattggattagttttaaaaaactgggaaaaaagtatgatttgtcttttgtttgaaagaagggaaaaggtatgatagttacttataactacagtatggaattatatttatttatctaattttaaattttaattctaagataatgatgtgtataaaaacaataatttgcgttttttttttaaatattcgatatattcaaagcatagtcataataaataatttttatttatttaacttgtgttttaaaatccacatgcactaacaaattatctttaagttattatatttatatacttaattattattatttttttcattttgatctttttcttcatttttcattccattatttataacctgtataaacttttctttctttagtatttgctctttctgtcttcccttcttccaccaatacatcccaaatttgggatatacgttgtttttctcccagttcttttataaagggaggagagacaaacttagtgctttaaaaatacacgtaacaaattctttgtcaatattatgtatgatagcaccgatagacctacttacgtcaacatgaaacagcaaagaaaattatgtaagagaaaaaagaccaagaacgaatttacaacgcacgcgtagcagattatattgtccacgtgttattgtttaatgggtcctggtgttacgtgtaaggcatttagggtgggcaaatgcatgtttttcttagctaattgccctgccaataagaagaggtgttcgcagtaagaaagataaactttaatacatgctcaaagtaaaattcttagttaatgatttatttttaatttaaatttaactcaacattttatatttatttataagatattatgattatatatttaatttcacactaagtatcgtgtttttagaatatagaataatctttttaagagacttaaaaattaaaaggttaactgttctaaaaaaatcattaaactaaaggagactaagaagggaaaattgaaatcatgaaagcaaattaaagaaacttgtctattgtatataactttttttgatacatgtctatattatataatattgaccaatttatttgctttattcttgataagataaactagactttcttgtaaaagataaccattgctttaattaggaggaccttatctcatggatgaggttgacatgtttgtgtgtatcatagaaatgatagacagaaatccagaattttaaaggacctatctcatgaatgaggttgacatgtttgtgtgtatcatagaaataaattcagaatttatttataaagatgagtttcatattacaaggagttttttttatatagaattgagaaaggaaacacacacaaactaagcagtagttcagctatttatactgattttttacaaataaacaactcactaatattagtaatttgttacaattgttttaactacaagcttagtttgttagaactattttaattaccaacttaatttgttacttatgtgaaccaacctatcaacaatttgcatatataggatatgattacgaaatttcagacgcattgtacactgtttataaccaaataacccaacaaggtttgatgaaagaaaaggaggagtacaaacaaaagaccaaagttgccaatcccaactgttgttgcctttgtggatcttggtgtgttaatcttatatataatatacacattcactttttaaattttttttattagtgcttaataattaatatccgattgatggtttattagtacaatttttaataattaatggtttattagtataatttttatttaatacaaaataaattattagtataggaatttccattaattctttctaggttggtcgagtatagaaatttccattaactatattctgaattttccttccctttctaaaagatctgcagtttcacacgagtgatcaaaggaatgggaaaaaaatgtaatagaaaattaccttagtttagtatttaatttttgaacaggcaacaactgttcatttcatgaaactcattttgcttaacgtggacaggttcacctagattacctcgatgcaggagcaaacataatattaacagcatcttatcaggtaattatcatattaattttttttttcatccctacaactctacattttaattttgccgtctttttggggttggggtgcaggccactattcaaggttttgaggccaaagggtaggtgaaactatgcttagaagaagtgtggagattgcacgtgaggcacgagaaatttattatgataggtgcaccaaagattcttctgactttatgagagatgaaagatataggaaacgtcccattttaattgcagcttctgtgggaagctatggagcgtatttggctgatggctctgaatatgtgtgagtgaacaaaaccaattatgtcaaaatagtcattaaagttggacttatgttgatttcaattaatattcactgttttgttactttttagtttgtagcataaatttttaacaactagttctgaattgcaaatataatttactaattgtatttgagtttaagatgaaaattttcatgattgaagtcaaaactgtacttccaaaataaagcaatgttgcagcaatatatatgacttaagtctacattgatttttctctcttcacagtggggactatggtgatgcagttactgtccagacactgaaagattttcacagggaaagagtaaagattcttgttgaggctggtgctgacttaatagcctttgaaacaattccaaataagctggaggcacaggtatttactaactaacaaacagactcacttatttgttacttgctttttatgtctgaaacagtaagaatctgtaatagaaatgttcaaaatgcagtgtcaattaccatttactaataccatagaaaattggaaattaccattgcatttttgtctagtttctccttgattttgagcaatcttattaattttcgttacaatttgataaataggcttatgctgaacttctcgaggaagaaggcatagaaactcctgcgtggttttcttttagttgtaaggatgaaagcaatgtggttagtggtgactctatctttgaatgcgcttcaatagctgattcatgcagacaagttgttgcggttggagttaattgtactgctcctagatttattcatggattgatttcatttatcaagaaggtgcaactttcaaataatactctgctctacactatcaaaatgtgctaattggcaatattgttttgaataacttgtgagttggccttctagttgattgtatactgtgcatgaaatgttctttaactagtgtctttaaggtactcgttgctagaagaccttataaactattctcaagtgagaaatgctaataacactaatttgtccgataacagctcactttatgacagaatttaacactccgtttttaaatagcaggcaacaagtaaaccagtacttgtatatcccaacagtggggagacttatatcgctgagagcaaccaatgggtggtgagttctgcttctctctttttacatggcctcagcttgtttttatgttcatgtttaaccaacttcaaatctaattccagttataataaatgatacttcctcatcaatttaaatgtctgaacctcatttttgcatgttttcaagtccttgttacgaatcttttcattgacattctataatttgcaacgtgaatttcgaaatataatctaaatgaagttactaaaaagcaaatcaacatgcacacattctgcatacactgccactttagtggtgtggacagaacactttttttttgttaaaccacaatgtgctataagaattcgtatatataattctagtttagtatcatcaaattgataacttaaaatttgtcttatagaaatcaagtggggcagcagagcatgattttgtctcctacataggcaagtggcgtgatgctggggcttccctttttggtggctgctgcaggactactcctaatactataagaggcatagcagaggcaacatatgggaaacttaaagacaaatgtatataa

SEQ ID NO: 17 - protein, 15 aa, synthetic construct
  VARIANT 5..14: note = X can be any amino acid
LLEFXXXXXXXXXXS

SEQ ID NO: 18 - protein, 6 aa, synthetic construct
NPSPYM

SEQ ID NO: 19 - RNA, 24 nt, synthetic construct
  source 1..24: mol_type = other RNA
gagtctgcagagcctagttatcat

SEQ ID NO: 20 - RNA, 24 nt, synthetic construct
  source 1..24: mol_type = other RNA
aggattctaccatcatcatcccca

SEQ ID NO: 21 - RNA, 24 nt, synthetic construct
  source 1..24: mol_type = other RNA
aggccaaagggttctctagagaag

SEQ ID NO: 22 - DNA, 24 bp, Glycine max
  source 1..24: mol_type = genomic DNA
gagtctgcagagcctagttatcat

SEQ ID NO: 23 - DNA, 24 bp, Glycine max
  source 1..24: mol_type = genomic DNA
aggattctaccatcatcatcccca

SEQ ID NO: 24 - DNA, 24 bp, Glycine max
  source 1..24: mol_type = genomic DNA
aggccaaagggttctctagagaag

SEQ ID NO: 25 - DNA, 3960 bp, synthetic construct
  source 1..3960: mol_type = other DNA
atggccctgttccaggacttcacccatctctacccactctcaaagaccatgcgcttcgagcttaagccaatcggaaagacccttgagcacatccacgccaagaactttttgtcccaggatgagactatggccgacatgtaccagaaggtgaaggctatcctcgatgactaccacagggatttcattgccgacatgatgggcgaagtgaagcttaccaagctcgccgagttctacgatgtgtacctcaagttccgcaagaacccaaaggatgatggactccagaagcagctcaaggatcttcaggctgtgctgcgcaaagagatcgttaagcctattggaaacggcggcaagtacaaggctggatacgatagacttttcggcgccaagcttttcaaggacggaaaagagcttggcgacctcgctaagttcgtgattgctcaagaaggcgagtcctctccaaagcttgctcatttggctcacttcgagaagttctccacctacttcaccggcttccacagaaaccgtaagaacatgtactccgacgaggataagcacaccgctattacctacaggctcatccacgagaacctgccacgcttcattgataacctccagatcctcgctaccatcaagcaaaagcactctgccctctacgaccagatcatcaacgagcttactgcctccggacttgatgtgtctcttgcttctcacctcgacggctaccataagcttttgacccaagagggcattaccgcctacaacactcttctcggaggaatttctggtgaggctggctctaggaagatccagggtattaacgaactcatcaactcccaccacaaccagcactgccataagtctgagaggattgctaagctcaggccactccacaagcagatcctttctgatggaatgggcgtgtccttcctgccatcaaagttcgctgatgactctgagatgtgccaggctgtgaacgagttctataggcactacgctgatgtgttcgccaaggtgcagtctctcttcgatggattcgatgaccaccaaaaggacggcatctacgtcgagcacaagaacctcaacgagttgtccaagcaggctttcggagatttcgctctccttggaagagtgctggatggctactatgtggatgttgtgaaccccgagttcaacgagagattcgctaaggctaagaccgataacgctaaggccaagctcaccaaagagaaggacaagttcatcaagggcgtgcactcactcgcttctctcgaacaagctattgagcactacaccgctaggcacgatgatgagtctgttcaggctggaaagctcggccaatatttcaagcacggacttgctggtgtggacaacccaattcagaagatccacaacaaccactccaccatcaagggattccttgagagagaaagaccagctggcgaaagggctctcccaaagattaagtctggaaagaacccagagatgacccagctcaggcagcttaaagagcttcttgacaacgctcttaacgtggcccacttcgctaagcttctcactaccaagaccactctcgataaccaggacggtaacttctacggtgagttcggtgctctctacgatgagcttgctaagatccccaccttgtacaacaaggtgagggactaccttagccagaagccattctctaccgagaagtacaagctcaacttcggcaacccaaccttgctcaacggatgggatctcaacaaagaaaaggataacttcgggatcatcctccagaaggacggttgctactaccttgctttgctcgataaggcccacaagaaggtgttcgataacgcaccaaacaccggcaagaacgtctaccagaagatgatctacaagctgctccccggaccaaacaagatgcttccaaaggtgttcttcgccaagtccaacctcgactactacaacccttctgctgagctgttggataagtacgctcagggcactcataagaagggcaacaacttcaacctcaaggactgccacgcactcatcgatttcttcaaggccggaatcaacaagcacccagagtggcaacatttcggcttcaagttctccccaaccagctcctaccaggatctctctgatttctacagagaggttgagccacagggctaccaggtgaagttcgtggatatcaacgccgactacatcaacgaacttgttgagcagggacagctctacctcttccagatctataacaaggacttcagccctaaggctcacggcaagccaaaccttcataccctctacttcaaggctctgttctccaaggacaacctcgcaaaccccatctacaagttgaacggcgaggctcagatcttctaccgcaaggcttctcttgacatgaacgagactaccatccacagagctggtgaggtgctcgaaaacaagaaccctgataaccccaagaaacgccagttcgtgtacgacatcatcaaggacaagaggtacacccaggataagttcatgctccacgtgccaatcaccatgaacttcggagttcagggcatgaccatcaaagagttcaacaagaaagtcaaccagagcatccagcagtacgacgaggttaacgtgatcggaattgatagaggtgagaggcaccttctctacctcaccgtgattaactccaagggcgagattctcgagcagcgctcccttaacgatattaccactgcttctgctaacggcacccagatgactactccataccacaagatcctcgacaagcgcgagattgagagactcaacgctagagttggatggggcgagatcgagactatcaaagagcttaagtccggctacctctctcacgttgtgcaccagatttcccagctcatgctcaagtacaacgctatcgtggtgcttgaggaccttaacttcggtttcaagcgcggaaggttcaaggtcgagaagcagatctaccaaaacttcgaaaacgccctcattaagaagctcaaccacctcgttctcaaggatgaggctgatgatgagatcggctcttacaagaacgctctccagctcactaacaactttaccgacctcaagtccatcggaaagcagaccggattcttgttctacgtgccagcttggaacacctccaagatcgatccagagactggattcgtggatctcctcaagccacgctacgagaacattgctcaatcccaggctttcttcggcaagttcgacaagatctgctacaacgctgacaaggactacttcgagttccacatcgactacgccaagttcaccgacaaggcaaagaactccaggcagatatggaagatctgcagtcacggcgacaagcgttacgtgtacgataagactgccaaccagaacaagggtgctaccaagggaatcaacgtgaacgacgagctgaagtcactcttcgctaggcatcacattaacgacaagcagcccaacctcgtgatggacatttgccagaacaacgacaaagaattccacaagtccctgatctacctcctcaagacccttcttgctctcaggtactccaacgcttcctccgatgaggatttcatcttgtccccagtggctaacgatgagggcatgttcttcaactccgctcttgctgatgatacccagccacaaaacgctgatgctaacggtgcttaccacattgctctcaaaggactttgggtcctcgagcagatcaagaactccgatgacctcaacaaggttaagctcgccattgacaaccagacctggttgaacttcgctcagaacaggaaaaggccggcggccacgaaaaaggccggccaggcaaaaaagaaaaagggatcctacccatacgatgttccagattacgcttatccctacgacgtgcctgattatgcatacccatatgatgtccccgactatgccggatccccaaagaaaaagcgcaaggtgtga

SEQ ID NO: 26 - protein, 1319 aa, synthetic construct
MALFQDFTHLYPLSKTMRFELKPIGKTLEHIHAKNFLSQDETMADMYQKVKAILDDYHRDFIADMMGEVKLTKLAEFYDVYLKFRKNPKDDGLQKQLKDLQAVLRKEIVKPIGNGGKYKAGYDRLFGAKLFKDGKELGDLAKFVIAQEGESSPKLAHLAHFEKFSTYFTGFHRNRKNMYSDEDKHTAITYRLIHENLPRFIDNLQILATIKQKHSALYDQIINELTASGLDVSLASHLDGYHKLLTQEGITAYNTLLGGISGEAGSRKIQGINELINSHHNQHCHKSERIAKLRPLHKQILSDGMGVSFLPSKFADDSEMCQAVNEFYRHYADVFAKVQSLFDGFDDHQKDGIYVEHKNLNELSKQAFGDFALLGRVLDGYYVDVVNPEFNERFAKAKTDNAKAKLTKEKDKFIKGVHSLASLEQAIEHYTARHDDESVQAGKLGQYFKHGLAGVDNPIQKIHNNHSTIKGFLERERPAGERALPKIKSGKNPEMTQLRQLKELLDNALNVAHFAKLLTTKTTLDNQDGNFYGEFGALYDELAKIPTLYNKVRDYLSQKPFSTEKYKLNFGNPTLLNGWDLNKEKDNFGIILQKDGCYYLALLDKAHKKVFDNAPNTGKNVYQKMIYKLLPGPNKMLPKVFFAKSNLDYYNPSAELLDKYAQGTHKKGNNFNLKDCHALIDFFKAGINKHPEWQHFGFKFSPTSSYQDLSDFYREVEPQGYQVKFVDINADYINELVEQGQLYLFQIYNKDFSPKAHGKPNLHTLYFKALFSKDNLANPIYKLNGEAQIFYRKASLDMNETTIHRAGEVLENKNPDNPKKRQFVYDIIKDKRYTQDKFMLHVPITMNFGVQGMTIKEFNKKVNQSIQQYDEVNVIGIDRGERHLLYLTVINSKGEILEQRSLNDITTASANGTQMTTPYHKILDKREIERLNARVGWGEIETIKELKSGYLSHVVHQISQLMLKYNAIVVLEDLNFGFKRGRFKVEKQIYQNFENALIKKLNHLVLKDEADDEIGSYKNALQLTNNFTDLKSIGKQTGFLFYVPAWNTSKIDPETGFVDLLKPRYENIAQSQAFFGKFDKICYNADKDYFEFHIDYAKFTDKAKNSRQIWKICSHGDKRYVYDKTANQNKGATKGINVNDELKSLFARHHINDKQPNLVMDICQNNDKEFHKSLIYLLKTLLALRYSNASSDEDFILSPVANDEGMFFNSALADDTQPQNADANGAYHIALKGLWVLEQIKNSDDLNKVKLAIDNQTWLNFAQNRKRPAATKKAGQAKKKKGSYPYDVPDYAYPYDVPDYAYPYDVPDYAGSPKKKRKV